European Patent Application EP 4 296 674 A1, published December 27, 2023. Title: INNOVATIVE MOLECULES DECREASING VIRULENCE OF MYCOBACTERIUM FOR THE TREATMENT OF TUBERCULOSIS. Applicant: Université Toulouse III - Paul Sabatier et al. The sequence listing filed with the application follows.

SEQUENCE LISTING (9 sequences)

SEQ ID NO: 1 - protein, 142 aa, Mycobacterium tuberculosis
MALREFSSVKVGDQLPEKTYPLTRQDLVNYAGVSGDLNPIHWDDEIAKVVGLDTAIAHGMLTMGIGGGYVTSWVGDPGAVTEYNVRFTAVVPVPNDGKGAELVFNGRVKSVDPESKSVTIALTATTGGKKIFGRAIASAKLA

SEQ ID NO: 2 - protein, 166 aa, Mycobacterium tuberculosis
MTVPEEAQTLIGKHYRAPDHFLVGREKIREFAVAVKDDHPTHYSEPDAAAAGYPALVAPLTFLAIAGRRVQLEIFTKFNIPINIARVFHRDQKFRFHRPILANDKLYFDTYLDSVIESHGTVLAEIRSEVTDAEGKPVVTSVVTMLGEAAHHEADADATVAAIASI

SEQ ID NO: 3 - protein, 219 aa, artificial
  Ntrp-HadB
MPEVVFSVDHSGSGTMYPYDVPDYASSVINFTGSSGPLVKVCGLQSTEAAECALDSDADLLGIICVPNRGGSGSGLKMALREFSSVKVGDQLPEKTYPLTRQDLVNYAGVSGDLNPIHWDDEIAKVVGLDTAIAHGMLTMGIGGGYVTSWVGDPGAVTEYNVRFTAVVPVPNDGKGAELVFNGRVKSVDPESKSVTIALTATTGGKKIFGRAIASAKLA

SEQ ID NO: 4 - protein, 386 aa, artificial
  HadD-Ctrp
MPEVVFSVDHSGSHHHHHHIEGRGSLKMTVPEEAQTLIGKHYRAPDHFLVGREKIREFAVAVKDDHPTHYSEPDAAAAGYPALVAPLTFLAIAGRRVQLEIFTKFNIPINIARVFHRDQKFRFHRPILANDKLYFDTYLDSVIESHGTVLAEIRSEVTDAEGKPVVTSVVTMLGEAAHHEADADATVAAIASIIDGSGSGGKRTIDPVIARKISSLVKAYKNSSGTPKYLVGVFRNQPKEDVLALVNDYGIDIVQLHGDESWQEYQEFLGLPVIKRLVFPKDCNILLSAASQKPHSFIPLFDSEAGGTGELLDWNSISDWVGRQESPESLHFMLAGGLTPENVGDALRLNGVIGVDVSGGVETNGVKDSNKIANFVKNAKKGSGKP

SEQ ID NO: 5 - protein, 172 aa, artificial
  Ntrp-Esat6
MPEVVFSVDHSGSGTMYPYDVPDYASSVINFTGSSGPLVKVCGLQSTEAAECALDSDADLLGIICVPNRGGSGSGLKMTEQQWNFAGIEAAASAIQGNVTSIHSLLDEGKQSLTKLAAAWGGSGSEAYQGVQQKWDATATELNNALQNLARTISEAGQAMASTEGNVTGMFA

SEQ ID NO: 6 - protein, 320 aa, artificial
  Cfp10-Ctrp
MPEVVFSVDHSGSHHHHHHIEGRGSLKMAEMKTDAATLAQEAGNFERISGDLKTQIDQVESTAGSLQGQWRGAAGTAAQAAVVRFQEAANKQKQELDEISTNIRQAGVQYSRADEEQQQALSSQMGFIDGSGSGGKRTIDPVIARKISSLVKAYKNSSGTPKYLVGVFRNQPKEDVLALVNDYGIDIVQLHGDESWQEYQEFLGLPVIKRLVFPKDCNILLSAASQKPHSFIPLFDSEAGGTGELLDWNSISDWVGRQESPESLHFMLAGGLTPENVGDALRLNGVIGVDVSGGVETNGVKDSNKIANFVKNAKKGSGKP

SEQ ID NO: 7 - protein, 386 aa, artificial
  HadC-Ctrp
MPEVVFSVDHSGSHHHHHHIEGRGSLKMALKTDIRGMIWRYPDYFIVGREQCREFARAVKCDHPAFFSEEAAADLGYDALVAPLTFVTILAKYVQLDFFRHVDVGMETMQIVQVDQRFVFHKPVLAGDKLWARMDIHSVDERFGADIVVTRNLCTNDDGELVMEAYTTLMGQQGDGSARLKWDKESGQVIRTAIDGSGSGGKRTIDPVIARKISSLVKAYKNSSGTPKYLVGVFRNQPKEDVLALVNDYGIDIVQLHGDESWQEYQEFLGLPVIKRLVFPKDCNILLSAASQKPHSFIPLFDSEAGGTGELLDWNSISDWVGRQESPESLHFMLAGGLTPENVGDALRLNGVIGVDVSGGVETNGVKDSNKIANFVKNAKKGSGKP

SEQ ID NO: 8 - protein, 44 aa, artificial
  N-terminal domain from Trp1p protein (Ntrp)
SSVINFTGSSGPLVKVCGLQSTEAAECALDSDADLLGIICVPNR

SEQ ID NO: 9 - protein, 185 aa, artificial
  C-terminal domain from Trp1p protein (Ctrp)
KRTIDPVIARKISSLVKAYKNSSGTPKYLVGVFRNQPKEDVLALVNDYGIDIVQLHGDESWQEYQEFLGLPVIKRLVFPKDCNILLSAASQKPHSFIPLFDSEAGGTGELLDWNSISDWVGRQESPESLHFMLAGGLTPENVGDALRLNGVIGVDVSGGVETNGVKDSNKIANFVKNAKKGSGKP